European Patent Specification EP 3 889 610 B1, published February 7, 2024. Title: BIOMARKER COMPOSITION FOR PREDICTING CANCER MALIGNANT PROGNOSIS INDUCED BY MICROPLASTIC EXPOSURE. Applicant: KOREA INSTITUTE OF RADIOLOGICAL & MEDICAL SCIENCES. The sequence listing filed with the application follows.

SEQUENCE LISTING (14 sequences)

SEQ ID NO: 1 - DNA, 24 bp, Artificial Sequence
  GAPDH Forward
gcctcaagatcatcagcaatgcct

SEQ ID NO: 2 - DNA, 24 bp, Artificial Sequence
  GAPDH Reverse
tgtggtcatgagtccttccacgat

SEQ ID NO: 3 - DNA, 21 bp, Artificial Sequence
  N-cadherin Forward
agaggcttctggtgaaatcgc

SEQ ID NO: 4 - DNA, 20 bp, Artificial Sequence
  N-cadherin Reverse
tggaaagcttctcacggcat

SEQ ID NO: 5 - DNA, 19 bp, Artificial Sequence
  CD44 Forward
ccaatgcctttgatggacc

SEQ ID NO: 6 - DNA, 21 bp, Artificial Sequence
  CD44 Reverse
tctgtctgtgctgtcggtgat

SEQ ID NO: 7 - DNA, 20 bp, Artificial Sequence
  PD-L1 Forward
ttgggaaatggaggataaga

SEQ ID NO: 8 - DNA, 21 bp, Artificial Sequence
  PD-L1 Reverse
ggatgtgccagaggtagttct

SEQ ID NO: 9 - DNA, 22 bp, Artificial Sequence
  NR1D1 Forward
ctggactccaacaacaacacag

SEQ ID NO: 10 - DNA, 20 bp, Artificial Sequence
  NR1D1 Reverse
ggggatggtgggaagtaggt

SEQ ID NO: 11 - DNA, 20 bp, Artificial Sequence
  NPAS2 Forward
gtatcacgcctctccttggg

SEQ ID NO: 12 - DNA, 20 bp, Artificial Sequence
  NPAS2 Reverse
attacaggaggggctaggca

SEQ ID NO: 13 - DNA, 23 bp, Artificial Sequence
  ACE2 Forward
cattggagcaagtgttggatctt

SEQ ID NO: 14 - DNA, 22 bp, Artificial Sequence
  ACE2 Reverse
gagctaatgcatgccattctca